European Patent Application EP 4 137 559 A1, published February 22, 2023. Title: Method of recovering extracellular vesicles. Applicant: H.U. Group Research Institute G.K. The sequence listing filed with the application follows.

SEQUENCE LISTING (3 sequences)

SEQ ID NO: 1 - DNA, 26 bp, Artificial Sequence
  Forward primer for detecting EML4-ALK mRNA
cagatgatagccgtaataaattgtcg

SEQ ID NO: 2 - DNA, 19 bp, Artificial Sequence
  Reverse primer for detecting EML4-ALK mRNA
cttccggcggtacacttgg

SEQ ID NO: 3 - DNA, 25 bp, Artificial Sequence
  Fluorescent probe for detecting EML4-ALK mRNA
actgcagacaagcataaagatgtca